European Patent Application EP 4 806 453 A1, published September 16, 2026. Title: Targeting opsin expression with mRNA therapy for myopia control and myopia treatment. Applicant: Carl Zeiss Vision International GmbH. Application EP. The sequence listing filed with the application follows.

SEQUENCE LISTING (3 sequences)

SEQ ID NO: 1 - DNA, 1242 bp, synthetic construct
  source 1..1242: mol_type = other DNA; note = cDNA sequence for human red opsin
gccagggccggctgccgtcggggacagggctttccatagccatggcccagcagtggagcctccaaaggctcgcaggccgccatccgcaggacagctatgaggacagcacccagtccagcatcttcacctacaccaacagcaactccaccagaggccccttcgaaggcccgaattaccacatcgctcccagatgggtgtaccacctcaccagtgtctggatgatctttgtggtcactgcatccgtcttcacaaatgggcttgtgctggcggccaccatgaagttcaagaagctgcgccacccgctgaactggatcctggtgaacctggcggtcgctgacctagcagagaccgtcatcgccagcactatcagcattgtgaaccaggtctctggctacttcgtgctgggccaccctatgtgtgtcctggagggctacaccgtctccctgtgtgggatcacaggtctctggtctctggccatcatttcctgggagagatggatggtggtctgcaagccctttggcaatgtgagatttgatgccaagctggccatcgtgggcattgccttctcctggatctgggctgctgtgtggacagccccgcccatctttggttggagcaggtactggccccacggcctgaagacttcatgcggcccagacgtgttcagcggcagctcgtaccccggggtgcagtcttacatgattgtcctcatggtcacctgctgcatcatcccactcgctatcatcatgctctgctacctccaagtgtggctggccatccgagcggtggcaaagcagcagaaagagtctgaatccacccagaaggcagagaaggaagtgacgcgcatggtggtggtgatgatctttgcgtactgcgtctgctggggaccctacaccttcttcgcatgctttgctgctgccaaccctggttacgccttccaccctttgatggctgccctgccggcctactttgccaaaagtgccactatctacaaccccgttatctatgtctttatgaaccggcagtttcgaaactgcatcttgcagcttttcgggaagaaggttgacgatggctctgaactctccagcgcctccaaaacggaggtctcatctgtgtcctcggtatcgcctgcatgaggtctgcctcctacccatcccgcccaccggggctttggccacctctcctttccccctccttctccatccctgtaaaataaatgtaatttatctttgccaaaaccaa

SEQ ID NO: 2 - DNA, 1106 bp, synthetic construct
  source 1..1106: mol_type = other DNA; note = cDNA sequence for human blue opsin
atccatgagaaaaatgtcggaggaagagttttatctgttcaaaaatatctcttcagtggggccgtgggatgggcctcagtaccacattgcccctgtctgggccttctacctccaggcagctttcatgggcactgtcttccttatagggttcccactcaatgccatggtgctggtggccacactgcgctacaaaaagttgcggcagcccctcaactacattctggtcaacgtgtccttcggaggcttcctcctctgcatcttctctgtcttccctgtcttcgtcgccagctgtaacggatacttcgtcttcggtcgccatgtttgtgctttggagggcttcctgggcactgtagcaggtctggttacaggatggtcactggccttcctggcctttgagcgctacattgtcatctgtaagcccttcggcaacttccgcttcagctccaagcatgcactgacggtggtcctggctacctggaccattggtattggcgtctccatcccacccttctttggctggagccggttcatccctgagggcctgcagtgttcctgtggccctgactggtacaccgtgggcaccaaataccgcagcgagtcctatacgtggttcctcttcatcttctgcttcattgtgcctctctccctcatctgcttctcctacactcagctgctgagggccctgaaagctgttgcagctcagcagcaggagtcagctacgacccagaaggctgaacgggaggtgagccgcatggtggttgtgatggtaggatccttctgtgtctgctacgtgccctacgcggccttcgccatgtacatggtcaacaaccgtaaccatgggctggacttacggcttgtcaccattccttcattcttctccaagagtgcttgcatctacaatcccatcatctactgcttcatgaataagcagttccaagcttgcatcatgaagatggtgtgtgggaaggccatgacagatgaatccgacacatgcagctcccagaaaacagaagtttctactgtctcgtctacccaagttggccccaactgaggacccaatattggcctgtttgcaacagctagaattaaattttacttttaagtaa

SEQ ID NO: 3 - DNA, 1998 bp, synthetic construct
  source 1..1998: mol_type = other DNA; note = cDNA sequence for human green opsin
cccactggccggtataaagcaccgtgaccctcaggtgacgcaccagggccggctgccgtcggggacagggctttccatagccatggcccagcagtggagcctccaaaggctcgcaggccgccatccgcaggacagctatgaggacagcacccagtccagcatcttcacctacaccaacagcaactccaccagaggccccttcgaaggcccgaattaccacatcgctcccagatgggtgtaccacctcaccagtgtctggatgatctttgtggtcattgcatccgtcttcacaaatgggcttgtgctggcggccaccatgaagttcaagaagctgcgccacccgctgaactggatcctggtgaacctggcggtcgctgacctggcagagaccgtcatcgccagcactatcagcgttgtgaaccaggtctatggctacttcgtgctgggccaccctatgtgtgtcctggagggctacaccgtctccctgtgtgggatcacaggtctctggtctctggccatcatttcctgggagagatggatggtggtctgcaagccctttggcaatgtgagatttgatgccaagctggccatcgtgggcattgccttctcctggatctgggctgctgtgtggacagccccgcccatctttggttggagcaggtactggccccacggcctgaagacttcatgcggcccagacgtgttcagcggcagctcgtaccccggggtgcagtcttacatgattgtcctcatggtcacctgctgcatcaccccactcagcatcatcgtgctctgctacctccaagtgtggctggccatccgagcggtggcaaagcagcagaaagagtctgaatccacccagaaggcagagaaggaagtgacgcgcatggtggtggtgatggtcctggcattctgcttctgctggggaccatacgccttcttcgcatgctttgctgctgccaaccctggctaccccttccaccctttgatggctgccctgccggccttctttgccaaaagtgccactatctacaaccccgttatctatgtctttatgaaccggcagtttcgaaactgcatcttgcagcttttcgggaagaaggttgacgatggctctgaactctccagcgcctccaaaacggaggtctcatctgtgtcctcggtatcgcctgcatgaggtctgcctcctacccatcccgcccaccggggctttggccacctctcctttccccctccttctccatccctgtaaaataaatgtaatttatctttgccaaaaccaacaaagtcacagaggctttcactgcagtgtgggaccacctgagcctctgcgtgtgcaggcactgggtctcgagagggtgcaagggggataaagaggagagagcgcttcatagactttaagttttcccgagcctcatgtctaccgatggcgtgaaaggatcctggcaaaacagaagtgtgaggcaggtgggcgtctatatccatttcaccaggctggtggttacataatcggcaagcaagagctgtggaggggcttgctggatgccctcagcacccaggaggagggagggagctagcaagctaaggcaggtggccctcctggccccttaaggtccatctgctggaggcccagagtccttggagtacagtctacacctggaggggacccattcctgccagtctgtggcagggatggcgcgccacctctgccaggccaggaccccaagcccgatcagcatcagcatggtgcaggtgcacaggcgtgagctgatcagtgacgaggggcaggcacacaaggtggagacaaagaccaagaggacggttgccagtgagaggcgcggactcaggaacttgaacaacatctgcgggggacggctttggaggtgctccgctgcctccagttgggtgacttgctgtagcatctccagcttggatattcggctcttgaaggtctccgtgatctcctgcaggagacgaaaatgcacgcaccagaagtca